European Patent Application EP 4 245 310 A1, published September 20, 2023. Title: Use of an enzyme fusion protein for prevention or treatment of neuropathy. Applicant: HANMI PHARM. CO., LTD. The sequence listing filed with the application follows.

SEQUENCE LISTING (15 sequences)

SEQ ID NO: 1 - DNA, 43 bp, Artificial Sequence
  Fc(S2P)_F
ctggcggtggcggatcgccaccatgcccagcacctgagttcct

SEQ ID NO: 2 - DNA, 43 bp, Artificial Sequence
  Fc(S2P)_R
aggaactcaggtgctgggcatggtggcgatccgccaccgccag

SEQ ID NO: 3 - DNA, 43 bp, Artificial Sequence
  Fc(N71Q)_F
agccgcgggaggagcagttccaaagcacgtaccgtgtggtcag

SEQ ID NO: 4 - DNA, 43 bp, Artificial Sequence
  Fc(N71Q)_R
ctgaccacacggtacgtgctttggaactgctcctcccgcggct

SEQ ID NO: 5 - DNA, 1287 bp, Homo sapiens
atgcagctgaggaacccagaactacatctgggctgcgcgcttgcgcttcgcttcctggccctcgtttcctgggacatccctggggctagagcactggacaatggattggcaaggacgcctaccatgggctggctgcactgggagcgcttcatgtgcaaccttgactgccaggaagagccagattcctgcatcagtgagaagctcttcatggagatggcagagctcatggtctcagaaggctggaaggatgcaggttatgagtacctctgcattgatgactgttggatggctccccaaagagattcagaaggcagacttcaggcagaccctcagcgctttcctcatgggattcgccagctagctaattatgttcacagcaaaggactgaagctagggatttatgcagatgttggaaataaaacctgcgcaggcttccctgggagttttggatactacgacattgatgcccagacctttgctgactggggagtagatctgctaaaatttgatggttgttactgtgacagtttggaaaatttggcagatggttataagcacatgtccttggccctgaataggactggcagaagcattgtgtactcctgtgagtggcctctttatatgtggccctttcaaaagcccaattatacagaaatccgacagtactgcaatcactggcgaaattttgctgacattgatgattcctggaaaagtataaagagtatcttggactggacatcttttaaccaggagagaattgttgatgttgctggaccagggggttggaatgacccagatatgttagtgattggcaactttggcctcagctggaatcagcaagtaactcagatggccctctgggctatcatggctgctcctttattcatgtctaatgacctccgacacatcagccctcaagccaaagctctccttcaggataaggacgtaattgccatcaatcaggaccccttgggcaagcaagggtaccagcttagacagggagacaactttgaagtgtgggaacgacctctctcaggcttagcctgggctgtagctatgataaaccggcaggagattggtggacctcgctcttataccatcgcagttgcttccctgggtaaaggagtggcctgtaatcctgcctgcttcatcacacagctcctccctgtgaaaaggaagctagggttctatgaatggacttcaaggttaagaagtcacataaatcccacaggcactgttttgcttcagctagaaaatacaatgcagatgtcattaaaagacttactt

SEQ ID NO: 6 - protein, 429 aa, Homo sapiens
MQLRNPELHLGCALALRFLALVSWDIPGARALDNGLARTPTMGWLHWERFMCNLDCQEEPDSCISEKLFMEMAELMVSEGWKDAGYEYLCIDDCWMAPQRDSEGRLQADPQRFPHGIRQLANYVHSKGLKLGIYADVGNKTCAGFPGSFGYYDIDAQTFADWGVDLLKFDGCYCDSLENLADGYKHMSLALNRTGRSIVYSCEWPLYMWPFQKPNYTEIRQYCNHWRNFADIDDSWKSIKSILDWTSFNQERIVDVAGPGGWNDPDMLVIGNFGLSWNQQVTQMALWAIMAAPLFMSNDLRHISPQAKALLQDKDVIAINQDPLGKQGYQLRQGDNFEVWERPLSGLAWAVAMINRQEIGGPRSYTIAVASLGKGVACNPACFITQLLPVKRKLGFYEWTSRLRSHINPTGTVLLQLENTMQMSLKDLL

SEQ ID NO: 7 - DNA, 666 bp, Artificial Sequence
  Fc varinat
ccaccatgcccagcacctgagttcctggggggaccatcagtcttcctgttccccccaaaacccaaggacaccctcatgatctcccggacccctgaggtcacatgcgtggtggtggacgtgagccaggaagaccctgaggtccagttcaactggtacgtggacggcgtggaggtgcataatgccaagacaaagccgcgggaggagcagttccaaagcacgtaccgtgtggtcagcgtcctcaccgtcctgcaccaggactggctgaatggcaaggagtacaagtgcaaggtctccaacaaaggcctcccatcctccatcgagaaaaccatctccaaagccaaagggcagccccgagaaccacaggtgtacaccctgcccccatcccaggaggagatgaccaagaaccaggtcagcctgacctgcctggtcaaaggcttctatcccagcgacatcgccgtggagtgggagagcaatgggcagccggagaacaactacaagaccacgcctcccgtgctggactccgacggctccttcttcctctacagcaggctaaccgtggacaagagcaggtggcaggaggggaacgtcttctcatgctccgtgatgcatgaggctctgcacaaccactacacgcagaagagcctctccctgtctctgggtaaatga

SEQ ID NO: 8 - protein, 221 aa, Artificial Sequence
  Fc variant
PSCPAPEFLGGPSVFLFPPKPKDTLMISRTPEVTCVVVDVSQEDPEVQFNWYVDGVEVHNAKTKPREEQFNSTYRVVSVLTVLHQDWLNGKEYKCKVSNKGLPSSIEKTISKAKGQPREPQVYTLPPSQEEMTKNQVSLTCLVKGFYPSDIAVEWESNGQPENNYKTTPPVLDSDGSFFLYSRLTVDKSRWQEGNVFSCSVMHEALHNHYTQKSLSLSLGK

SEQ ID NO: 9 - protein, 221 aa, Artificial Sequence
  Fc varinat
PPCPAPEFLGGPSVFLFPPKPKDTLMISRTPEVTCVVVDVSQEDPEVQFNWYVDGVEVHNAKTKPREEQFQSTYRVVSVLTVLHQDWLNGKEYKCKVSNKGLPSSIEKTISKAKGQPREPQVYTLPPSQEEMTKNQVSLTCLVKGFYPSDIAVEWESNGQPENNYKTTPPVLDSDGSFFLYSRLTVDKSRWQEGNVFSCSVMHEALHNHYTQKSLSLSLGK

SEQ ID NO: 10 - DNA, 90 bp, Artificial Sequence
  peptide linker
ggcggcggaggttcaggtggtggtggctctggcggtggagggtcggggggaggcggctctggaggagggggctccggtgggggaggtagc

SEQ ID NO: 11 - protein, 30 aa, Artificial Sequence
  peptide linker
GGGGSGGGGSGGGGSGGGGSGGGGSGGGGS

SEQ ID NO: 12 - DNA, 2043 bp, Artificial Sequence
  alpha galactosidase-Fc fusion protein
atgcagctgaggaacccagaactacatctgggctgcgcgcttgcgcttcgcttcctggccctcgtttcctgggacatccctggggctagagcactggacaatggattggcaaggacgcctaccatgggctggctgcactgggagcgcttcatgtgcaaccttgactgccaggaagagccagattcctgcatcagtgagaagctcttcatggagatggcagagctcatggtctcagaaggctggaaggatgcaggttatgagtacctctgcattgatgactgttggatggctccccaaagagattcagaaggcagacttcaggcagaccctcagcgctttcctcatgggattcgccagctagctaattatgttcacagcaaaggactgaagctagggatttatgcagatgttggaaataaaacctgcgcaggcttccctgggagttttggatactacgacattgatgcccagacctttgctgactggggagtagatctgctaaaatttgatggttgttactgtgacagtttggaaaatttggcagatggttataagcacatgtccttggccctgaataggactggcagaagcattgtgtactcctgtgagtggcctctttatatgtggccctttcaaaagcccaattatacagaaatccgacagtactgcaatcactggcgaaattttgctgacattgatgattcctggaaaagtataaagagtatcttggactggacatcttttaaccaggagagaattgttgatgttgctggaccagggggttggaatgacccagatatgttagtgattggcaactttggcctcagctggaatcagcaagtaactcagatggccctctgggctatcatggctgctcctttattcatgtctaatgacctccgacacatcagccctcaagccaaagctctccttcaggataaggacgtaattgccatcaatcaggaccccttgggcaagcaagggtaccagcttagacagggagacaactttgaagtgtgggaacgacctctctcaggcttagcctgggctgtagctatgataaaccggcaggagattggtggacctcgctcttataccatcgcagttgcttccctgggtaaaggagtggcctgtaatcctgcctgcttcatcacacagctcctccctgtgaaaaggaagctagggttctatgaatggacttcaaggttaagaagtcacataaatcccacaggcactgttttgcttcagctagaaaatacaatgcagatgtcattaaaagacttacttggcggcggaggttcaggtggtggtggctctggcggtggagggtcggggggaggcggctctggaggagggggctccggtgggggaggtagcccaccatgcccagcacctgagttcctggggggaccatcagtcttcctgttccccccaaaacccaaggacaccctcatgatctcccggacccctgaggtcacatgcgtggtggtggacgtgagccaggaagaccctgaggtccagttcaactggtacgtggacggcgtggaggtgcataatgccaagacaaagccgcgggaggagcagttccaaagcacgtaccgtgtggtcagcgtcctcaccgtcctgcaccaggactggctgaatggcaaggagtacaagtgcaaggtctccaacaaaggcctcccatcctccatcgagaaaaccatctccaaagccaaagggcagccccgagaaccacaggtgtacaccctgcccccatcccaggaggagatgaccaagaaccaggtcagcctgacctgcctggtcaaaggcttctatcccagcgacatcgccgtggagtgggagagcaatgggcagccggagaacaactacaagaccacgcctcccgtgctggactccgacggctccttcttcctctacagcaggctaaccgtggacaagagcaggtggcaggaggggaacgtcttctcatgctccgtgatgcatgaggctctgcacaaccactacacgcagaagagcctctccctgtctctgggtaaatga

SEQ ID NO: 13 - protein, 680 aa, Artificial Sequence
  alpha galactosidase-Fc fusion protein
MQLRNPELHLGCALALRFLALVSWDIPGARALDNGLARTPTMGWLHWERFMCNLDCQEEPDSCISEKLFMEMAELMVSEGWKDAGYEYLCIDDCWMAPQRDSEGRLQADPQRFPHGIRQLANYVHSKGLKLGIYADVGNKTCAGFPGSFGYYDIDAQTFADWGVDLLKFDGCYCDSLENLADGYKHMSLALNRTGRSIVYSCEWPLYMWPFQKPNYTEIRQYCNHWRNFADIDDSWKSIKSILDWTSFNQERIVDVAGPGGWNDPDMLVIGNFGLSWNQQVTQMALWAIMAAPLFMSNDLRHISPQAKALLQDKDVIAINQDPLGKQGYQLRQGDNFEVWERPLSGLAWAVAMINRQEIGGPRSYTIAVASLGKGVACNPACFITQLLPVKRKLGFYEWTSRLRSHINPTGTVLLQLENTMQMSLKDLLGGGGSGGGGSGGGGSGGGGSGGGGSGGGGSPPCPAPEFLGGPSVFLFPPKPKDTLMISRTPEVTCVVVDVSQEDPEVQFNWYVDGVEVHNAKTKPREEQFQSTYRVVSVLTVLHQDWLNGKEYKCKVSNKGLPSSIEKTISKAKGQPREPQVYTLPPSQEEMTKNQVSLTCLVKGFYPSDIAVEWESNGQPENNYKTTPPVLDSDGSFFLYSRLTVDKSRWQEGNVFSCSVMHEALHNHYTQKSLSLSLGK

SEQ ID NO: 14 - protein, 12 aa, Homo sapiens
ESKYGPPCPSCP

SEQ ID NO: 15 - protein, 4 aa, Artificial Sequence
  Hinge region
PPCP